European Patent Application EP 4 309 651 A1, published January 24, 2024. Title: A therapeutic agent for hypertrophic cardiomyopathy. Applicant: JUNTENDO EDUCATIONAL FOUNDATION. The sequence listing filed with the application follows.

SEQUENCE LISTING (2 sequences)

SEQ ID NO: 1 - DNA, 25 bp, Artificial Sequence
catgtttgctctgatctgacacgca

SEQ ID NO: 2 - DNA, 25 bp, Artificial Sequence
cctcctacctcagttacaatttata